European Patent Specification EP 3 307 304 B1, published May 8, 2024. Title: Immunoglobulin fusion proteins and uses thereof. Applicant: UBI Pharma Inc WANG, Chang-Yi. Application PCT/US2016/036915. The sequence listing filed with the application follows.

SEQUENCE LISTING (74 sequences)

SEQ ID NO: 1 - protein, 15 aa, Homo sapiens
  SITE (1)..(15): wild type IgG1 hinge peptide sequence
EPKSCDKTHTCPPCP

SEQ ID NO: 2 - protein, 15 aa, Artificial Sequence
  Mutated IgG1 Hinge Region
  SITE (1)..(15): Artificial mutated IgG1 hinge peptide sequence
  SITE (5)..(5): S or G or T or A or V or L or I or M or deletion
  SITE (11)..(11): S or G or T or A or V or L or I or M or deletion
  SITE (14)..(14): S or G or T or A or V or L or I or M or deletion
EPKSXDKTHTXPPXP

SEQ ID NO: 3 - protein, 13 aa, Artificial Sequence
  Mutated IgG1 Hinge Region
  SITE (1)..(13): Artificial mutated IgG1 hinge peptide sequence
  SITE (5)..(5): S or G or T or A or V or L or I or M or deletion
  SITE (11)..(11): S or G or T or A or V or L or I or M or deletion
EPKSXDKTHTXPP

SEQ ID NO: 4 - protein, 10 aa, Artificial Sequence
  Mutated IgG1 Hinge Region
  SITE (1)..(10): Artificial mutated IgG1 hinge peptide sequence
  SITE (5)..(5): S or G or T or A or V or L or I or M or deletion
EPKSXDKTHT

SEQ ID NO: 5 - protein, 10 aa, Artificial Sequence
  Mutated IgG1 Hinge Region
  SITE (1)..(10): Artificial mutated IgG1 hinge peptide sequence
  SITE (6)..(6): S or G or T or A or V or L or I or M or deletion
  SITE (9)..(9): S or G or T or A or V or L or I or M or deletion
DKTHTXPPXP

SEQ ID NO: 6 - protein, 12 aa, Homo sapiens
  SITE (1)..(12): Wild type IgG2 hinge peptide sequence
ERKCCVECPPCP

SEQ ID NO: 7 - protein, 12 aa, Artificial Sequence
  Mutated IgG2 Hinge Region
  SITE (1)..(12): Artificial mutated IgG2 hinge peptide sequence
  SITE (4)..(4): S or G or T or A or V or L or I or M or deletion
  SITE (5)..(5): S or G or T or A or V or L or I or M or deletion
  SITE (8)..(8): S or G or T or A or V or L or I or M or deletion
  SITE (11)..(11): S or G or T or A or V or L or I or M or deletion
ERKXXVEXPPXP

SEQ ID NO: 8 - protein, 10 aa, Artificial Sequence
  Mutated IgG2 Hinge Region
  SITE (1)..(10): Artificial mutated IgG2 hinge peptide sequence
  SITE (4)..(4): S or G or T or A or V or L or I or M or deletion
  SITE (5)..(5): S or G or T or A or V or L or I or M or deletion
  SITE (8)..(8): S or G or T or A or V or L or I or M or deletion
ERKXXVEXPP

SEQ ID NO: 9 - protein, 7 aa, Artificial Sequence
  Mutated IgG2 Hinge Region
  SITE (1)..(7): Artificial mutated IgG2 hinge peptide sequence
  SITE (3)..(3): S or G or T or A or V or L or I or M or deletion
  SITE (6)..(6): S or G or T or A or V or L or I or M or deletion
VEXPPXP

SEQ ID NO: 10 - protein, 17 aa, Homo sapiens
  SITE (1)..(17): Wild type IgG3 hinge peptide sequence
ELKTPLGDTTHTCPRCP

SEQ ID NO: 11 - protein, 17 aa, Artificial Sequence
  Mutated IgG3 Hinge Region
  SITE (1)..(17): Artificial mutated IgG3 hinge peptide sequence
  SITE (13)..(13): S or G or T or A or V or L or I or M or deletion
  SITE (16)..(16): S or G or T or A or V or L or I or M or deletion
ELKTPLGDTTHTXPRXP

SEQ ID NO: 12 - protein, 15 aa, Artificial Sequence
  Mutated IgG3 Hinge Region
  SITE (1)..(15): Artificial mutated IgG3 hinge peptide sequence
  SITE (13)..(13): S or G or T or A or V or L or I or M or deletion
ELKTPLGDTTHTXPR

SEQ ID NO: 13 - protein, 12 aa, Artificial Sequence
  Mutated IgG3 Hinge Region
  SITE (1)..(12): Artificial mutated IgG3 hinge peptide sequence
ELKTPLGDTTHT

SEQ ID NO: 14 - protein, 15 aa, Homo sapiens
  SITE (1)..(15): Wild type IgG3 hinge peptide sequence
EPKSCDTPPPCPRCP

SEQ ID NO: 15 - protein, 15 aa, Artificial Sequence
  Mutated IgG3 Hinge Region
  SITE (1)..(15): Artificial mutated IgG3 hinge peptide sequence
  SITE (5)..(5): S or G or T or A or V or L or I or M or deletion
  SITE (11)..(11): S or G or T or A or V or L or I or M or deletion
  SITE (14)..(14): S or G or T or A or V or L or I or M or deletion
EPKSXDTPPPXPRXP

SEQ ID NO: 16 - protein, 13 aa, Artificial Sequence
  Mutated IgG3 Hinge Region
  SITE (1)..(13): Artificial mutated IgG3 hinge peptide sequence
  SITE (5)..(5): S or G or T or A or V or L or I or M or deletion
  SITE (11)..(11): S or G or T or A or V or L or I or M or deletion
EPKSXDTPPPXPR

SEQ ID NO: 17 - protein, 10 aa, Artificial Sequence
  Mutated IgG3 Hinge Region
  SITE (1)..(10): Artificial mutated IgG3 hinge peptide sequence
  SITE (5)..(5): S or G or T or A or V or L or I or M or deletion
EPKSXDTPPP

SEQ ID NO: 18 - protein, 10 aa, Artificial Sequence
  Mutated IgG3 Hinge Region
  SITE (1)..(10): Artificial mutated IgG3 hinge peptide sequence
  SITE (6)..(6): S or G or T or A or V or L or I or M or deletion
  SITE (9)..(9): S or G or T or A or V or L or I or M or deletion
DTPPPXPRXP

SEQ ID NO: 19 - protein, 12 aa, Homo sapiens
  SITE (1)..(12): Wild type IgG4 hinge peptide sequence
ESKYGPPCPSCP

SEQ ID NO: 20 - protein, 12 aa, Artificial Sequence
  Mutated IgG4 Hinge Region
  SITE (1)..(12): Artificial mutated IgG4 hinge peptide sequence
  SITE (10)..(10): S or G or T or A or V or L or I or M or deletion
EXKYGPPCPXCP

SEQ ID NO: 21 - protein, 9 aa, Artificial Sequence
  Mutated IgG4 Hinge Region
  SITE (1)..(9): Artificial mutated IgG4 hinge peptide sequence
  SITE (2)..(2): S or G or T or A or V or L or I or M or deletion
EXKYGPPCP

SEQ ID NO: 22 - protein, 10 aa, Artificial Sequence
  Mutated IgG4 Hinge Region
  SITE (1)..(10): Artificial mutated IgG4 hinge peptide sequence
  SITE (8)..(8): S or G or T or A or V or L or I or M or deletion
KYGPPCPXCP

SEQ ID NO: 23 - protein, 15 aa, Artificial Sequence
  Mutated IgG Hinge Region
  SITE (1)..(15): Artificial IgG1 hinge peptide sequence
EPKSSDKTHTSPPSP

SEQ ID NO: 24 - protein, 13 aa, Artificial Sequence
  Mutated IgG Hinge Region
  SITE (1)..(13): Artificial IgG1 hinge peptide sequence
EPKSSDKTHTSPP

SEQ ID NO: 25 - protein, 14 aa, Artificial Sequence
  Mutated IgG Hinge Region
  SITE (1)..(14): Artificial IgG1 hinge peptide sequence
EPKSSDKTHTSPPP

SEQ ID NO: 26 - protein, 10 aa, Artificial Sequence
  Mutated IgG Hinge Region
  SITE (1)..(10): Artificial IgG1 hinge peptide sequence
EPKSSDKTHT

SEQ ID NO: 27 - protein, 10 aa, Artificial Sequence
  Mutated IgG Hinge Region
  SITE (1)..(10): Artificial IgG1 hinge peptide sequence
DKTHTSPPSP

SEQ ID NO: 28 - protein, 8 aa, Homo sapiens
  SITE (1)..(8): Artificial IgG1 hinge peptide sequence
DKTHTSPP

SEQ ID NO: 29 - protein, 12 aa, Artificial Sequence
  Mutated IgG Hinge Region
  SITE (1)..(12): Artificial IgG1 hinge peptide sequence
EPKSDKTHTPPP

SEQ ID NO: 30 - protein, 14 aa, Artificial Sequence
  Mutated IgG Hinge Region
  SITE (1)..(14): Artificial IgG1 hinge peptide sequence
EPKSDKTHTSPPSP

SEQ ID NO: 31 - protein, 15 aa, Artificial Sequence
  Mutated IgG Hinge Region
  SITE (1)..(15): Artificial IgG1 hinge peptide sequence
EPKSGDKTHTGPPGP

SEQ ID NO: 32 - protein, 13 aa, Artificial Sequence
  Mutated IgG Hinge Region
  SITE (1)..(13): Artificial IgG1 hinge peptide sequence
EPKSGDKTHTGPP

SEQ ID NO: 33 - protein, 14 aa, Artificial Sequence
  Mutated IgG Hinge Region
  SITE (1)..(14): Artificial IgG1 hinge peptide sequence
EPKSGDKTHTGPPP

SEQ ID NO: 34 - protein, 10 aa, Artificial Sequence
  Mutated IgG Hinge Region
  SITE (1)..(10): Artificial IgG1 hinge peptide sequence
EPKSGDKTHT

SEQ ID NO: 35 - protein, 10 aa, Artificial Sequence
  Mutated IgG Hinge Region
  SITE (1)..(10): Artificial IgG1 hinge peptide sequence
DKTHTGPPGP

SEQ ID NO: 36 - protein, 8 aa, Artificial Sequence
  Mutated IgG Hinge Region
  SITE (1)..(8): Artificial IgG1 hinge peptide sequence
DKTHTGPP

SEQ ID NO: 37 - protein, 14 aa, Artificial Sequence
  Mutated IgG Hinge Region
  SITE (1)..(14): Artificial IgG1 hinge peptide sequence
EPKSDKTHTGPPGP

SEQ ID NO: 38 - protein, 15 aa, Artificial Sequence
  Mutated IgG Hinge Region
  SITE (1)..(15): Artificial IgG1 hinge peptide sequence
EPKSGDKTHTSPPSP

SEQ ID NO: 39 - protein, 15 aa, Artificial Sequence
  Mutated IgG Hinge Region
  SITE (1)..(15): Artificial IgG1 hinge peptide sequence
EPKSGDKTHTGPPSP

SEQ ID NO: 40 - protein, 15 aa, Artificial Sequence
  Mutated IgG Hinge Region
  SITE (1)..(15): Artificial IgG1 hinge peptide sequence
EPKSSDKTHTGPPGP

SEQ ID NO: 41 - protein, 15 aa, Artificial Sequence
  Mutated IgG Hinge Region
  SITE (1)..(15): Artificial IgG1 hinge peptide sequence
EPKSSDKTHTGPPSP

SEQ ID NO: 42 - protein, 13 aa, Artificial Sequence
  Mutated IgG Hinge Region
  SITE (1)..(13): Artificial IgG1 hinge peptide sequence
EPKSSDKTHTGPP

SEQ ID NO: 43 - protein, 13 aa, Homo sapiens
  SITE (1)..(13): Artificial IgG1 hinge peptide sequence
EPKSGDKTHTSPP

SEQ ID NO: 44 - protein, 15 aa, Artificial Sequence
  Mutated IgG Hinge Region
  SITE (1)..(15): Artificial IgG1 hinge peptide sequence
EPKSTDKTHTTPPTP

SEQ ID NO: 45 - protein, 13 aa, Artificial Sequence
  Mutated IgG Hinge Region
  SITE (1)..(13): Artificial IgG1 hinge peptide sequence
EPKSTDKTHTTPP

SEQ ID NO: 46 - protein, 14 aa, Artificial Sequence
  Mutated IgG Hinge Region
  SITE (1)..(14): Artificial IgG1 hinge peptide sequence
EPKSTDKTHTTPPP

SEQ ID NO: 47 - protein, 10 aa, Artificial Sequence
  Mutated IgG Hinge Region
  SITE (1)..(10): Artificial IgG1 hinge peptide sequence
EPKSTDKTHT

SEQ ID NO: 48 - protein, 10 aa, Artificial Sequence
  Mutated IgG Hinge Region
  SITE (1)..(10): Artificial IgG1 hinge peptide sequence
DKTHTTPPTP

SEQ ID NO: 49 - protein, 8 aa, Artificial Sequence
  Mutated IgG Hinge Region
  SITE (1)..(8): Artificial IgG1 hinge peptide sequence
DKTHTTPP

SEQ ID NO: 50 - protein, 14 aa, Artificial Sequence
  Mutated IgG Hinge Region
  SITE (1)..(14): Artificial IgG1 hinge peptide sequence
EPKSDKTHTTPPTP

SEQ ID NO: 51 - protein, 15 aa, Artificial Sequence
  Mutated IgG Hinge Region
  SITE (1)..(15): Artificial IgG1 hinge peptide sequence
EPKSSDKTHTTPPTP

SEQ ID NO: 52 - protein, 15 aa, Artificial Sequence
  Mutated IgG Hinge Region
  SITE (1)..(15): Artificial IgG1 hinge peptide sequence
EPKSSDKTHTSPPTP

SEQ ID NO: 53 - protein, 15 aa, Artificial Sequence
  Mutated IgG Hinge Region
  SITE (1)..(15): Artificial IgG1 hinge peptide sequence
EPKSADKTHTLPPMP

SEQ ID NO: 54 - protein, 15 aa, Artificial Sequence
  Mutated IgG Hinge Region
  SITE (1)..(15): Artificial IgG1 hinge peptide sequence
EPKSVDKTHTLPPIP

SEQ ID NO: 55 - protein, 15 aa, Artificial Sequence
  Mutated IgG Hinge Region
  SITE (1)..(15): Artificial IgG1 hinge peptide sequence
EPKSLDKTHTAPPAP

SEQ ID NO: 56 - protein, 13 aa, Artificial Sequence
  Mutated IgG Hinge Region
  SITE (1)..(13): Artificial IgG1 hinge peptide sequence
EPKSVDKTHTAPP

SEQ ID NO: 57 - protein, 13 aa, Artificial Sequence
  Mutated IgG Hinge Region
  SITE (1)..(13): Artificial IgG1 hinge peptide sequence
EPKSMDKTHTVPP

SEQ ID NO: 58 - protein, 13 aa, Artificial Sequence
  Mutated IgG Hinge Region
  SITE (1)..(13): Artificial IgG1 hinge peptide sequence
EPKSIDKTHTLPP

SEQ ID NO: 59 - protein, 10 aa, Artificial Sequence
  Mutated IgG Hinge Region
  SITE (1)..(10): Artificial IgG1 hinge peptide sequence
DKTHTAPPLP

SEQ ID NO: 60 - protein, 10 aa, Artificial Sequence
  Mutated IgG Hinge Region
  SITE (1)..(10): Artificial IgG1 hinge peptide sequence
DKTHTVPPLP

SEQ ID NO: 61 - protein, 216 aa, Homo sapiens
  SITE (1)..(216): Fc region of wild type IgG1 (CH2-CH3 domain of human IgG1)
APELLGGPSVFLFPPKPKDTLMISRTPEVTCVVVDVSHEDPEVKFNWYVDGVEVHNAKTKPREEQYNSTYRVVSVLTVLHQDWLNGKEYKCKVSNKALPAPIEKTISKAKGQPREPQVYTLPPSRDELTKNQVSLTCLVKGFYPSDIAVEWESNGQPENNYKTTPPVLDSDGSFFLYSKLTVDKSRWQQGNVFSCSVMHEALHNHYTQKSLSLSPG

SEQ ID NO: 62 - protein, 216 aa, Artificial Sequence
  Fc region of human IgG1 with glycosylation site mutated from Asn to His
  SITE (67)..(67): Glycosylation site at residue 67 in wild type sequence mutated to His
APELLGGPSVFLFPPKPKDTLMISRTPEVTCVVVDVSHEDPEVKFNWYVDGVEVHNAKTKPREEQYHSTYRVVSVLTVLHQDWLNGKEYKCKVSNKALPAPIEKTISKAKGQPREPQVYTLPPSRDELTKNQVSLTCLVKGFYPSDIAVEWESNGQPENNYKTTPPVLDSDGSFFLYSKLTVDKSRWQQGNVFSCSVMHEALHNHYTQKSLSLSPG

SEQ ID NO: 63 - protein, 216 aa, Artificial Sequence
  Fc region of human IgG1 with glycosylation site mutated from Asn to Ala
  SITE (67)..(67): Glycosylation site at residue 67 in wild type sequence mutated to Ala
APELLGGPSVFLFPPKPKDTLMISRTPEVTCVVVDVSHEDPEVKFNWYVDGVEVHNAKTKPREEQYASTYRVVSVLTVLHQDWLNGKEYKCKVSNKALPAPIEKTISKAKGQPREPQVYTLPPSRDELTKNQVSLTCLVKGFYPSDIAVEWESNGQPENNYKTTPPVLDSDGSFFLYSKLTVDKSRWQQGNVFSCSVMHEALHNHYTQKSLSLSPG

SEQ ID NO: 64 - protein, 216 aa, Artificial Sequence
  Fc region of human IgG1 with variable residues at the wild type glycosylation site
  SITE (67)..(67): N or H or A
  SITE (67)..(67): Glycosylation site in wild-type IgG1
APELLGGPSVFLFPPKPKDTLMISRTPEVTCVVVDVSHEDPEVKFNWYVDGVEVHNAKTKPREEQYXSTYRVVSVLTVLHQDWLNGKEYKCKVSNKALPAPIEKTISKAKGQPREPQVYTLPPSRDELTKNQVSLTCLVKGFYPSDIAVEWESNGQPENNYKTTPPVLDSDGSFFLYSKLTVDKSRWQQGNVFSCSVMHEALHNHYTQKSLSLSPG

SEQ ID NO: 65 - protein, 193 aa, Homo sapiens
  SITE (1)..(193): Human EPO protein
MGVHECPAWLWLLLSLLLSLPLGLPVLGAPPRLICDSRVLERYLLEAKEAENITTGCAEHCSLNENITVPDTKVNFYAWKRMEVGQQAVEVWQGLALLSEAVLRGGALLVNSSQPWEPLQLHVDKAVSGLGSLTTLRALGAQKEAISPPDAASAAPLRTITADTFRKLFRVYSNFLRGKLKLYTGEACRTGDR

SEQ ID NO: 66 - protein, 419 aa, Artificial Sequence
  Erythropoietin Single Chain Fc Fusion Protein (EPO-sFc)
  SITE (1)..(419): Erythropoietin single chain Fc Fusion Protein (EPO-sFc)
  SITE (1)..(193): Erythropoietin (EPO)
  SITE (194)..(203): Mutated Hinge Region
  SITE (204)..(419): Single Chain Fc Region (sFc)
MGVHECPAWLWLLLSLLLSLPLGLPVLGAPPRLICDSRVLERYLLEAKEAENITTGCAEHCSLNENITVPDTKVNFYAWKRMEVGQQAVEVWQGLALLSEAVLRGGALLVNSSQPWEPLQLHVDKAVSGLGSLTTLRALGAQKEAISPPDAASAAPLRTITADTFRKLFRVYSNFLRGKLKLYTGEACRTGDRDKTHTSPPSPAPELLGGPSVFLFPPKPKDTLMISRTPEVTCVVVDVSHEDPEVKFNWYVDGVEVHNAKTKPREEQYHSTYRVVSVLTVLHQDWLNGKEYKCKVSNKALPAPIEKTISKAKGQPREPQVYTLPPSRDELTKNQVSLTCLVKGFYPSDIAVEWESNGQPENNYKTTPPVLDSDGSFFLYSKLTVDKSRWQQGNVFSCSVMHEALHNHYTQKSLSLSPG

SEQ ID NO: 67 - protein, 461 aa, Homo sapiens [sequence omitted]

SEQ ID NO: 68 - protein, 692 aa, Artificial Sequence
  Factor IX Single Chain Fc Fusion Protein (FIX-sFc)
  SITE (1)..(692): Factor IX single chain Fc Fusion Protein (FIX-sFc)
  SITE (1)..(461): Factor IX (FIX)
  SITE (462)..(476): Mutated Hinge Region
  SITE (477)..(692): single chain Fc Region (sFc)
MQRVNMIMAESPGLITICLLGYLLSAECTVFLDHENANKILNRPKRYNSGKLEEFVQGNLERECMEEKCSFEEAREVFENTERTTEFWKQYVDGDQCESNPCLNGGSCKDDINSYECWCPFGFEGKNCELDVTCNIKNGRCEQFCKNSADNKVVCSCTEGYRLAENQKSCEPAVPFPCGRVSVSQTSKLTRAEAVFPDVDYVNSTEAETILDNITQSTQSFNDFTRVVGGEDAKPGQFPWQVVLNGKVDAFCGGSIVNEKWIVTAAHCVETGVKITVVAGEHNIEETEHTEQKRNVIRIIPHHNYNAAINKYNHDIALLELDEPLVLNSYVTPICIADKEYTNIFLKFGSGYVSGWGRVFHKGRSALVLQYLRVPLVDRATCLRSTKFTIYNNMFCAGFHEGGRDSCQGDSGGPHVTEVEGTSFLTGIISWGEECAMKGKYGIYTKVSRYVNWIKEKTKLTEPKSSDKTHTSPPSPAPELLGGPSVFLFPPKPKDTLMISRTPEVTCVVVDVSHEDPEVKFNWYVDGVEVHNAKTKPREEQYHSTYRVVSVLTVLHQDWLNGKEYKCKVSNKALPAPIEKTISKAKGQPREPQVYTLPPSRDELTKNQVSLTCLVKGFYPSDIAVEWESNGQPENNYKTTPPVLDSDGSFFLYSKLTVDKSRWQQGNVFSCSVMHEALHNHYTQKSLSLSPG

SEQ ID NO: 69 - protein, 189 aa, Homo sapiens
  SITE (1)..(189): Interferon alpha 8 (IFNa8)
MALTFYLLVALVVLSYKSFSSLGCDLPQTHSLGNRRALILLAQMRRISPFSCLKDRHDFEFPQEEFDDKQFQKAQAISVLHEMIQQTFNLFSTKDSSAALDETLLDEFYIELDQQLNDLESCVMQEVGVIESPLMYEDSILAVRKYFQRITLYLTEKKYSSCAWEVVRAEIMRSFSLSINLQKRLKSKE

SEQ ID NO: 70 - protein, 420 aa, Artificial Sequence
  Interferon alpha single chain fusion protein (IFNa-sFc)
  SITE (1)..(189): Interferon alpha (IFNa)
  SITE (1)..(204): Hinge Region
  SITE (205)..(420): single chain Fc region (sFc)
MALTFYLLVALVVLSYKSFSSLGCDLPQTHSLGNRRALILLAQMRRISPFSCLKDRHDFEFPQEEFDDKQFQKAQAISVLHEMIQQTFNLFSTKDSSAALDETLLDEFYIELDQQLNDLESCVMQEVGVIESPLMYEDSILAVRKYFQRITLYLTEKKYSSCAWEVVRAEIMRSFSLSINLQKRLKSKEEPKSSDKTHTSPPSPAPELLGGPSVFLFPPKPKDTLMISRTPEVTCVVVDVSHEDPEVKFNWYVDGVEVHNAKTKPREEQYHSTYRVVSVLTVLHQDWLNGKEYKCKVSNKALPAPIEKTISKAKGQPREPQVYTLPPSRDELTKNQVSLTCLVKGFYPSDIAVEWESNGQPENNYKTTPPVLDSDGSFFLYSKLTVDKSRWQQGNVFSCSVMHEALHNHYTQKSLSLSPG

SEQ ID NO: 71 - protein, 204 aa, Homo sapiens
  SITE (1)..(204): Granulocyte-Colony Stimulating Factor (GCSF)
MAGPATQSPMKLMALQLLLWHSALWTVQEATPLGPASSLPQSFLLKCLEQVRKIQGDGAALQEKLCATYKLCHPEELVLLGHSLGIPWAPLSSCPSQALQLAGCLSQLHSGLFLYQGLLQALEGISPELGPTLDTLQLDVADFATTIWQQMEELGMAPALQPTQGAMPAFASAFQRRAGGVLVASHLQSFLEVSYRVLRHLAQP

SEQ ID NO: 72 - protein, 435 aa, Artificial Sequence
  Granulocyte-Colony Stimulating Factor single chaing Fc Fusion Protein (GCSF-sFc)
  SITE (1)..(204): Granulocyte-Colony Stimulating Factor (GCSF)
  SITE (205)..(219): Mutated Hinge Region
  SITE (220)..(435): Single chain Fc (sFc)
MAGPATQSPMKLMALQLLLWHSALWTVQEATPLGPASSLPQSFLLKCLEQVRKIQGDGAALQEKLCATYKLCHPEELVLLGHSLGIPWAPLSSCPSQALQLAGCLSQLHSGLFLYQGLLQALEGISPELGPTLDTLQLDVADFATTIWQQMEELGMAPALQPTQGAMPAFASAFQRRAGGVLVASHLQSFLEVSYRVLRHLAQPEPKSSDKTHTSPPSPAPELLGGPSVFLFPPKPKDTLMISRTPEVTCVVVDVSHEDPEVKFNWYVDGVEVHNAKTKPREEQYHSTYRVVSVLTVLHQDWLNGKEYKCKVSNKALPAPIEKTISKAKGQPREPQVYTLPPSRDELTKNQVSLTCLVKGFYPSDIAVEWESNGQPENNYKTTPPVLDSDGSFFLYSKLTVDKSRWQQGNVFSCSVMHEALHNHYTQKSLSLSPG

SEQ ID NO: 73 - protein, 187 aa, Homo sapiens
  SITE (1)..(187): Interferon beta (IFNb)
MNNRWILHAAFLLCFSTTALSMSYNLLGFLQRSSNFQCQKLLWQLNGRLEYCLKDRMNFDIPEEIKQLQQFQKEDAALTIYEMLQNIFAIFRQDSSSTGWNETIVENLLANVYHQINHLKTVLEEKLEKEDFTRGKLMSSLHLKRYYGRILHYLKAKEYSHCAWTIVRVEILRNFYFINRLTGYLRN

SEQ ID NO: 74 - protein, 419 aa, Artificial Sequence
  Interferon beta single chain Fc Fusion Protein (IFNb-sFc)
  SITE (1)..(187): Interferon beta (IFNb)
  SITE (188)..(202): Mutated Hinge Region
  SITE (203)..(419): Single chain Fc (sFc)
MNNRWILHAAFLLCFSTTALSMSYNLLGFLQRSSNFQCQKLLWQLNGRLEYCLKDRMNFDIPEEIKQLQQFQKEDAALTIYEMLQNIFAIFRQDSSSTGWNETIVENLLANVYHQINHLKTVLEEKLEKEDFTRGKLMSSLHLKRYYGRILHYLKAKEYSHCAWTIVRVEILRNFYFINRLTGYLRNEPKSSDKTHTSPPSPAPELLGGPSVFLFPPKPKDTLMISRTPEVTCVVVDVSHEDPEVKFNWYVDGVEVHNAKTKPREEQYASTYRVVSVLTVLHQDWLNGKEYKCKVSNKALPAPIEKTISKAKGQPREPQVYTLPPSRDELTKNQVSLTCLVKGFYPSDIAVEWESNGQPENNYKTTPPVLDSDGSFFLYSKLTVDKSRWQQGNVFSCSVMHEALHNHYTQKSLSLSPGK